European Patent Application EP 4 273 171 A1, published November 8, 2023. Title: ANTIBODY CAPABLE OF BINDING TO TROP2, AND USE THEREOF. Applicant: NONA BIOSCIENCES (SUZHOU) CO., LTD. The sequence listing filed with the application follows.

SEQUENCE LISTING (293 sequences)

SEQ ID NO: 1 - protein, 25 aa, Artificial sequence
  Heavy chain variable region FR1
QVQLQESGPGLVKPSGTLSLTCAVS

SEQ ID NO: 2 - protein, 25 aa, Artificial sequence
  Heavy chain variable region FR1
QVELVESGGGVVQPGRSLRLSCGAS

SEQ ID NO: 3 - protein, 25 aa, Artificial sequence
  Heavy chain variable region FR1
QVNLVESGGGVVQPGRSLKLSCAAS

SEQ ID NO: 4 - protein, 25 aa, Artificial sequence
  Heavy chain variable region FR1
QVQLVESGGGVVQPGRSLRVSCIAS

SEQ ID NO: 5 - protein, 25 aa, Artificial sequence
  Heavy chain variable region FR1
QVQLQESGPRLVKPSETLSLTCAVS

SEQ ID NO: 6 - protein, 25 aa, Artificial sequence
  Heavy chain variable region FR1
QVQLVESGGGVVQPGRSLRLSCAAS

SEQ ID NO: 7 - protein, 25 aa, Artificial sequence
  Heavy chain variable region FR1
QVQLVESGGGVVQPGRSLRVSCAAS

SEQ ID NO: 8 - protein, 25 aa, Artificial sequence
  Heavy chain variable region FR1
QVQLVESGGGVVQPEKSLRLSCAAS

SEQ ID NO: 9 - protein, 25 aa, Artificial sequence
  Heavy chain variable region FR1
QVQLVESGGAVVQPGRSLRLSCAAS

SEQ ID NO: 10 - protein, 25 aa, Artificial sequence
  Heavy chain variable region FR1
QVQLVESGGGVVQPGRSLRLSCEAS

SEQ ID NO: 11 - protein, 25 aa, Artificial sequence
  Heavy chain variable region FR1
QVQLVQSGGGVVQPGRSLRLSCAAS

SEQ ID NO: 12 - protein, 25 aa, Artificial sequence
  Heavy chain variable region FR1
QVQLVESGGGVVQPGRSLRLSCEGS

SEQ ID NO: 13 - protein, 25 aa, Artificial sequence
  Heavy chain variable region FR1
QVQLVESGGGVVQPGRSLRLSCVAS

SEQ ID NO: 14 - protein, 25 aa, Artificial sequence
  Heavy chain variable region FR1
QVQLVESGGGVVQPGTSLRLSCVAS

SEQ ID NO: 15 - protein, 25 aa, Artificial sequence
  Heavy chain variable region FR1
QVQLVESGGDVVQPGRSLRLSCEAS

SEQ ID NO: 16 - protein, 25 aa, Artificial sequence
  Heavy chain variable region FR1
QVQLQQSGPGLVKPSQTLSLTCAIS

SEQ ID NO: 17 - protein, 25 aa, Artificial sequence
  Heavy chain variable region FR1
QVQLQESGPGLVKPSETLSLTCAVS

SEQ ID NO: 18 - protein, 25 aa, Artificial sequence
  Heavy chain variable region FR1
QVQLVESGGGVVQPGRSLRLSCATS

SEQ ID NO: 19 - protein, 8 aa, Artificial sequence
  Heavy chain variable region CDR1
GGSISSSN

SEQ ID NO: 20 - protein, 8 aa, Artificial sequence
  Heavy chain variable region CDR1
GDSISSHN

SEQ ID NO: 21 - protein, 7 aa, Artificial sequence
  Heavy chain variable region CDR1
GFTFSSY

SEQ ID NO: 22 - protein, 7 aa, Artificial sequence
  Heavy chain variable region CDR1
GFFFSSY

SEQ ID NO: 23 - protein, 8 aa, Artificial sequence
  Heavy chain variable region CDR1
GYSISSGY

SEQ ID NO: 24 - protein, 7 aa, Artificial sequence
  Heavy chain variable region CDR1
GFTFSSF

SEQ ID NO: 25 - protein, 8 aa, Artificial sequence
  Heavy chain variable region CDR1
GDSISSNN

SEQ ID NO: 26 - protein, 7 aa, Artificial sequence
  Heavy chain variable region CDR1
GFIFSTY

SEQ ID NO: 27 - protein, 7 aa, Artificial sequence
  Heavy chain variable region CDR1
GFTFSHY

SEQ ID NO: 28 - protein, 7 aa, Artificial sequence
  Heavy chain variable region CDR1
GFTFSND

SEQ ID NO: 29 - protein, 9 aa, Artificial sequence
  Heavy chain variable region CDR1
GDSVSSTSA

SEQ ID NO: 30 - protein, 7 aa, Artificial sequence
  Heavy chain variable region CDR1
GFIFSSY

SEQ ID NO: 31 - protein, 8 aa, Artificial sequence
  Heavy chain variable region CDR1
GYSINSGY

SEQ ID NO: 32 - protein, 19 aa, Artificial sequence
  Heavy chain variable region FR2
WWSWVRQPPGKGLEWIGEI

SEQ ID NO: 33 - protein, 19 aa, Artificial sequence
  Heavy chain variable region FR2
NMYWVRQAPGKGLEWVAGI

SEQ ID NO: 34 - protein, 19 aa, Artificial sequence
  Heavy chain variable region FR2
GMHWVRQAPGKGLEWVALI

SEQ ID NO: 35 - protein, 19 aa, Artificial sequence
  Heavy chain variable region FR2
GMHWVRQAPGKGLEWVAVI

SEQ ID NO: 36 - protein, 19 aa, Artificial sequence
  Heavy chain variable region FR2
YWGWIRQSPGMGLEWIAYI

SEQ ID NO: 37 - protein, 19 aa, Artificial sequence
  Heavy chain variable region FR2
GMQWVRQGPGKGLEWVAVM

SEQ ID NO: 38 - protein, 19 aa, Artificial sequence
  Heavy chain variable region FR2
GMQWVRQGPGKGLEWVAIM

SEQ ID NO: 39 - protein, 19 aa, Artificial sequence
  Heavy chain variable region FR2
GMHWVRQAPGKGLEWVAFI

SEQ ID NO: 40 - protein, 19 aa, Artificial sequence
  Heavy chain variable region FR2
GMHWVRQVPGKGLEWVAVI

SEQ ID NO: 41 - protein, 19 aa, Artificial sequence
  Heavy chain variable region FR2
GMHWVRQAPGMGLEWVAIM

SEQ ID NO: 42 - protein, 19 aa, Artificial sequence
  Heavy chain variable region FR2
GMHWVRQAPGKGLEWVAVV

SEQ ID NO: 43 - protein, 19 aa, Artificial sequence
  Heavy chain variable region FR2
VWNWIRQSPSRGLEWLGRT

SEQ ID NO: 44 - protein, 19 aa, Artificial sequence
  Heavy chain variable region FR2
FWAWIRQPPGKGLEWIGSI

SEQ ID NO: 45 - protein, 19 aa, Artificial sequence
  Heavy chain variable region FR2
GMHWVRQAPGKGLDWVAVI

SEQ ID NO: 46 - protein, 19 aa, Artificial sequence
  Heavy chain variable region FR2
FWAWIRQPPGMGLEWIGSI

SEQ ID NO: 47 - protein, 5 aa, Artificial sequence
  Heavy chain variable region CDR2
FHSGT

SEQ ID NO: 48 - protein, 5 aa, Artificial sequence
  Heavy chain variable region CDR2
YHSGI

SEQ ID NO: 49 - protein, 6 aa, Artificial sequence
  Heavy chain variable region CDR2
WDDGNN

SEQ ID NO: 50 - protein, 6 aa, Artificial sequence
  Heavy chain variable region CDR2
WSDGTN

SEQ ID NO: 51 - protein, 6 aa, Artificial sequence
  Heavy chain variable region CDR2
WYDGSN

SEQ ID NO: 52 - protein, 5 aa, Artificial sequence
  Heavy chain variable region CDR2
YHDGS

SEQ ID NO: 53 - protein, 6 aa, Artificial sequence
  Heavy chain variable region CDR2
WFDGSN

SEQ ID NO: 54 - protein, 5 aa, Artificial sequence
  Heavy chain variable region CDR2
YPGGN

SEQ ID NO: 55 - protein, 6 aa, Artificial sequence
  Heavy chain variable region CDR2
WYDGIK

SEQ ID NO: 56 - protein, 6 aa, Artificial sequence
  Heavy chain variable region CDR2
WYDGIM

SEQ ID NO: 57 - protein, 6 aa, Artificial sequence
  Heavy chain variable region CDR2
WFDGGS

SEQ ID NO: 58 - protein, 7 aa, Artificial sequence
  Heavy chain variable region CDR2
CYRSKWY

SEQ ID NO: 59 - protein, 5 aa, Artificial sequence
  Heavy chain variable region CDR2
YHSGR

SEQ ID NO: 60 - protein, 41 aa, Artificial sequence
  Heavy chain variable region FR3
TYYNPSLKSRVTILVDKSKNQFSLKLSSVTAADTAVYYCAR

SEQ ID NO: 61 - protein, 41 aa, Artificial sequence
  Heavy chain variable region FR3
TSYNPSLKSRVTISVDKSKNQFSLKLNSVTAADTAMYYCAR

SEQ ID NO: 62 - protein, 41 aa, Artificial sequence
  Heavy chain variable region FR3
KYYANSVKGRFTISRDNSKNTLYLQMNSLRTEDTALYYCAK

SEQ ID NO: 63 - protein, 41 aa, Artificial sequence
  Heavy chain variable region FR3
RYYTESVKGRFTISRDNSKNTLSLQMKSLRAEDTAVYYCAK

SEQ ID NO: 64 - protein, 41 aa, Artificial sequence
  Heavy chain variable region FR3
EDYVDSVKGRFTISRDNSKNTLYLQMNSLRGEDTAMYYCAR

SEQ ID NO: 65 - protein, 41 aa, Artificial sequence
  Heavy chain variable region FR3
TYCNPSLKSRVTMSVDTSKNQFSLKLRSVTAADTAVYYCAR

SEQ ID NO: 66 - protein, 41 aa, Artificial sequence
  Heavy chain variable region FR3
KYYVDSVKGRFTISRDNSKNTLYLQMNSLRAEDTAVYYCAR

SEQ ID NO: 67 - protein, 41 aa, Artificial sequence
  Heavy chain variable region FR3
PNYNPSLKSRVTISVDKSKNQFSLKLNSVTAADTAVYYCAR

SEQ ID NO: 68 - protein, 41 aa, Artificial sequence
  Heavy chain variable region FR3
EDYVDSVKGRFTISRDNSKNTLYLQMNSLRGEDTAVYYCAR

SEQ ID NO: 69 - protein, 41 aa, Artificial sequence
  Heavy chain variable region FR3
RYYPESVKGRFTISRDDSRNTVSLQMNSLRPEDTAVYYCAR

SEQ ID NO: 70 - protein, 41 aa, Artificial sequence
  Heavy chain variable region FR3
RYYVESVKGRFTISRDNSKNTLYLQMNRLRAEDTAVYYCAR

SEQ ID NO: 71 - protein, 41 aa, Artificial sequence
  Heavy chain variable region FR3
KDYVESVKGRFTISRDNSKNTLYLQMNRLRAEDTAVYYCAR

SEQ ID NO: 72 - protein, 41 aa, Artificial sequence
  Heavy chain variable region FR3
SYYVESVKGRFTISRDNSKNTLYLQMDRLRAEDTAVYYCAR

SEQ ID NO: 73 - protein, 41 aa, Artificial sequence
  Heavy chain variable region FR3
TDYNPSLKSRVIISVDKSKNQFSLKVRSVTAADTAVYYCAR

SEQ ID NO: 74 - protein, 41 aa, Artificial sequence
  Heavy chain variable region FR3
KYYIESVKGRFIISRDNSKNTLYLQMNRLRAEDTAVYYCAR

SEQ ID NO: 75 - protein, 41 aa, Artificial sequence
  Heavy chain variable region FR3
KYYVESVKGRFTISRDNSKNTLYLQMNRLRAEDTAVYYCAR

SEQ ID NO: 76 - protein, 41 aa, Artificial sequence
  Heavy chain variable region FR3
KNYVDSLKGRFTISRDNSKNTLYLQMNSLRAEDTAVYYCAR

SEQ ID NO: 77 - protein, 41 aa, Artificial sequence
  Heavy chain variable region FR3
KYYVESVKGRFTISRDNSKNTLNLQMNRLRAEDTAVYYCAR

SEQ ID NO: 78 - protein, 41 aa, Artificial sequence
  Heavy chain variable region FR3
TNYVESVKGRFTISRDNSKNTLNLQMNRLRAEDTAVYYCAR

SEQ ID NO: 79 - protein, 41 aa, Artificial sequence
  Heavy chain variable region FR3
KNYIESVKGRFTISRDNSKNTLYLQMNRLRAEDTAVYYCAR

SEQ ID NO: 80 - protein, 41 aa, Artificial sequence
  Heavy chain variable region FR3
KYYADSVKGRFTISRDNSKNTLYLQMNNLRAEDTAVYYCAR

SEQ ID NO: 81 - protein, 41 aa, Artificial sequence
  Heavy chain variable region FR3
NDYAVSVKSRITITPDTSKNQFSLRLNPVTPEDTAVYYCAR

SEQ ID NO: 82 - protein, 41 aa, Artificial sequence
  Heavy chain variable region FR3
TYYVESVKGRFTISRDNSKNTLNLQMNRLRAEDTAVYYCAR

SEQ ID NO: 83 - protein, 41 aa, Artificial sequence
  Heavy chain variable region FR3
THYNPSLKSRVIISLDTSKNQFSLKLRSVTAADSAVYYCAR

SEQ ID NO: 84 - protein, 41 aa, Artificial sequence
  Heavy chain variable region FR3
KYYADSVKGRFTISRDNSKNTLYLQMNSLRVEDTAVYYCAR

SEQ ID NO: 85 - protein, 41 aa, Artificial sequence
  Heavy chain variable region FR3
KNYVESVKGRFTISRDNSKNTLNLQMNRLRAEDTAVYYCAR

SEQ ID NO: 86 - protein, 11 aa, Artificial sequence
  Heavy chain variable region CDR3
DNTKSWDHFDH

SEQ ID NO: 87 - protein, 10 aa, Artificial sequence
  Heavy chain variable region CDR3
GSGVISYFDY

SEQ ID NO: 88 - protein, 12 aa, Artificial sequence
  Heavy chain variable region CDR3
DGWGSYGEYFQH

SEQ ID NO: 89 - protein, 12 aa, Artificial sequence
  Heavy chain variable region CDR3
DGWGTYGEYFQH

SEQ ID NO: 90 - protein, 12 aa, Artificial sequence
  Heavy chain variable region CDR3
GGYNSGWWAFDI

SEQ ID NO: 91 - protein, 9 aa, Artificial sequence
  Heavy chain variable region CDR3
DGAAAPFDY

SEQ ID NO: 92 - protein, 11 aa, Artificial sequence
  Heavy chain variable region CDR3
LDFSGWPLIDY

SEQ ID NO: 93 - protein, 12 aa, Artificial sequence
  Heavy chain variable region CDR3
GGYNSGWWAFDV

SEQ ID NO: 94 - protein, 14 aa, Artificial sequence
  Heavy chain variable region CDR3
DGGFGESNYYGLDV

SEQ ID NO: 95 - protein, 14 aa, Artificial sequence
  Heavy chain variable region CDR3
DGGFGELNYYGLDV

SEQ ID NO: 96 - protein, 7 aa, Artificial sequence
  Heavy chain variable region CDR3
DNWGFDY

SEQ ID NO: 97 - protein, 14 aa, Artificial sequence
  Heavy chain variable region CDR3
DGGFGELNYYGMDV

SEQ ID NO: 98 - protein, 13 aa, Artificial sequence
  Heavy chain variable region CDR3
DHPHYLGSGSFDY

SEQ ID NO: 99 - protein, 7 aa, Artificial sequence
  Heavy chain variable region CDR3
GDFRFDS

SEQ ID NO: 100 - protein, 9 aa, Artificial sequence
  Heavy chain variable region CDR3
EGYASGSYY

SEQ ID NO: 101 - protein, 12 aa, Artificial sequence
  Heavy chain variable region CDR3
ETSSWYVGYLQH

SEQ ID NO: 102 - protein, 11 aa, Artificial sequence
  Heavy chain variable region FR4
WGQGTLVTVSS

SEQ ID NO: 103 - protein, 11 aa, Artificial sequence
  Heavy chain variable region FR4
WGQGTMVTVSS

SEQ ID NO: 104 - protein, 11 aa, Artificial sequence
  Heavy chain variable region FR4
WGQGTTVTVSS

SEQ ID NO: 105 - protein, 23 aa, Artificial sequence
  Light chain variable region FR1
EIVLTQSPATLSLSPGERATLSC

SEQ ID NO: 106 - protein, 23 aa, Artificial sequence
  Light chain variable region FR1
DIQMTQSPSTLSASVGDRVTITC

SEQ ID NO: 107 - protein, 23 aa, Artificial sequence
  Light chain variable region FR1
DIQMTQSPSSLSASLGDRVTITC

SEQ ID NO: 108 - protein, 23 aa, Artificial sequence
  Light chain variable region FR1
DIQMTQSPSSLSASVGERVTITC

SEQ ID NO: 109 - protein, 23 aa, Artificial sequence
  Light chain variable region FR1
DIQMTQSPSSLSASVGDRVTITC

SEQ ID NO: 110 - protein, 23 aa, Artificial sequence
  Light chain variable region FR1
QVVMTQSPATLSVSPGERATLSC

SEQ ID NO: 111 - protein, 23 aa, Artificial sequence
  Light chain variable region FR1
EIVMTQSPATLSVSPGERATLSC

SEQ ID NO: 112 - protein, 23 aa, Artificial sequence
  Light chain variable region FR1
DIQLTQSPSFLSASVGDRVTITC

SEQ ID NO: 113 - protein, 23 aa, Artificial sequence
  Light chain variable region FR1
EIVLTQFPGTLSLSPGERATLSC

SEQ ID NO: 114 - protein, 23 aa, Artificial sequence
  Light chain variable region FR1
EIVMTQSPATLSVSPGERVSLSC

SEQ ID NO: 115 - protein, 11 aa, Artificial sequence
  Light chain variable region CDR1
RASQSVGSYLA

SEQ ID NO: 116 - protein, 11 aa, Artificial sequence
  Light chain variable region CDR1
RASQSIGNWLA

SEQ ID NO: 117 - protein, 11 aa, Artificial sequence
  Light chain variable region CDR1
RATQGISNYLA

SEQ ID NO: 118 - protein, 11 aa, Artificial sequence
  Light chain variable region CDR1
RASQNINSYLS

SEQ ID NO: 119 - protein, 11 aa, Artificial sequence
  Light chain variable region CDR1
RASQNINSYLH

SEQ ID NO: 120 - protein, 11 aa, Artificial sequence
  Light chain variable region CDR1
RASQGISHFLA

SEQ ID NO: 121 - protein, 11 aa, Artificial sequence
  Light chain variable region CDR1
RASQSISNWLA

SEQ ID NO: 122 - protein, 11 aa, Artificial sequence
  Light chain variable region CDR1
RASQSVSSKLA

SEQ ID NO: 123 - protein, 11 aa, Artificial sequence
  Light chain variable region CDR1
RASQSIGHWLA

SEQ ID NO: 124 - protein, 11 aa, Artificial sequence
  Light chain variable region CDR1
RASQSVSSNLA

SEQ ID NO: 125 - protein, 11 aa, Artificial sequence
  Light chain variable region CDR1
RASQSINSYLH

SEQ ID NO: 126 - protein, 11 aa, Artificial sequence
  Light chain variable region CDR1
RASQGINSYLG

SEQ ID NO: 127 - protein, 11 aa, Artificial sequence
  Light chain variable region CDR1
RASQGISSYLG

SEQ ID NO: 128 - protein, 12 aa, Artificial sequence
  Light chain variable region CDR1
RSSQSVSSSYLA

SEQ ID NO: 129 - protein, 11 aa, Artificial sequence
  Light chain variable region CDR1
RASQSVSSYLA

SEQ ID NO: 130 - protein, 11 aa, Artificial sequence
  Light chain variable region CDR1
RASQGISSYLA

SEQ ID NO: 131 - protein, 11 aa, Artificial sequence
  Light chain variable region CDR1
RSSQSVNNYLA

SEQ ID NO: 132 - protein, 11 aa, Artificial sequence
  Light chain variable region CDR1
RASQSVNGNVA

SEQ ID NO: 133 - protein, 11 aa, Artificial sequence
  Light chain variable region CDR1
RSSQSVNSYLA

SEQ ID NO: 134 - protein, 15 aa, Artificial sequence
  Light chain variable region FR2
WYQQKPGQAPSLLIY

SEQ ID NO: 135 - protein, 15 aa, Artificial sequence
  Light chain variable region FR2
WYQQKPGKAPKLLIY

SEQ ID NO: 136 - protein, 15 aa, Artificial sequence
  Light chain variable region FR2
WYQQKPGKVPNLLIY

SEQ ID NO: 137 - protein, 15 aa, Artificial sequence
  Light chain variable region FR2
WYQQKPGKVPKLLIY

SEQ ID NO: 138 - protein, 15 aa, Artificial sequence
  Light chain variable region FR2
WYQQKPGKAPKVLIY

SEQ ID NO: 139 - protein, 15 aa, Artificial sequence
  Light chain variable region FR2
WYQQKPGQAPRLIIY

SEQ ID NO: 140 - protein, 15 aa, Artificial sequence
  Light chain variable region FR2
WYQQKPGQAPRLLIY

SEQ ID NO: 141 - protein, 15 aa, Artificial sequence
  Light chain variable region FR2
WYQRKPGKAPKLLIY

SEQ ID NO: 142 - protein, 15 aa, Artificial sequence
  Light chain variable region FR2
WYQQKPGQAPRLLIS

SEQ ID NO: 143 - protein, 15 aa, Artificial sequence
  Light chain variable region FR2
WFQQKPGQAPRLLIY

SEQ ID NO: 144 - protein, 7 aa, Artificial sequence
  Light chain variable region CDR2
DASNRAT

SEQ ID NO: 145 - protein, 7 aa, Artificial sequence
  Light chain variable region CDR2
KASSLES

SEQ ID NO: 146 - protein, 7 aa, Artificial sequence
  Light chain variable region CDR2
AASTLQS

SEQ ID NO: 147 - protein, 7 aa, Artificial sequence
  Light chain variable region CDR2
AASSLQN

SEQ ID NO: 148 - protein, 7 aa, Artificial sequence
  Light chain variable region CDR2
AASSLQS

SEQ ID NO: 149 - protein, 7 aa, Artificial sequence
  Light chain variable region CDR2
GASTRAT

SEQ ID NO: 150 - protein, 7 aa, Artificial sequence
  Light chain variable region CDR2
IASTLQS

SEQ ID NO: 151 - protein, 7 aa, Artificial sequence
  Light chain variable region CDR2
VASTLQS

SEQ ID NO: 152 - protein, 7 aa, Artificial sequence
  Light chain variable region CDR2
GASSRAT

SEQ ID NO: 153 - protein, 7 aa, Artificial sequence
  Light chain variable region CDR2
DSSTRAT

SEQ ID NO: 154 - protein, 7 aa, Artificial sequence
  Light chain variable region CDR2
AASTRAT

SEQ ID NO: 155 - protein, 32 aa, Artificial sequence
  Light chain variable region FR3
GIPARFSGSGSGTDFTLTISSLEPEDFAVYYC

SEQ ID NO: 156 - protein, 32 aa, Artificial sequence
  Light chain variable region FR3
GVPSRFSGSGSGTEFTLTISSLQPDDFATYYC

SEQ ID NO: 157 - protein, 32 aa, Artificial sequence
  Light chain variable region FR3
GVPSRFSGSGSGTDLTLTISSLQPEDVATYYC

SEQ ID NO: 158 - protein, 32 aa, Artificial sequence
  Light chain variable region FR3
GVPSRFSGSGSGTDFTLTISSLQPEDFATYYC

SEQ ID NO: 159 - protein, 32 aa, Artificial sequence
  Light chain variable region FR3
GVPSRFSGSGSGTDFTLTISSLQPEDFAIYYC

SEQ ID NO: 160 - protein, 32 aa, Artificial sequence
  Light chain variable region FR3
GVPSRFSGSGSGTDFTLTISSLQPEDVATYYC

SEQ ID NO: 161 - protein, 32 aa, Artificial sequence
  Light chain variable region FR3
GVPSRFSGSGSGTEFTLTINSLQPDDFATYYC

SEQ ID NO: 162 - protein, 32 aa, Artificial sequence
  Light chain variable region FR3
GIPARFSGSGSGTEFTLTISSLQSEDFAVYYC

SEQ ID NO: 163 - protein, 32 aa, Artificial sequence
  Light chain variable region FR3
GVPSRFRGSGSGTEFTLTISSLQPDDFATYYC

SEQ ID NO: 164 - protein, 32 aa, Artificial sequence
  Light chain variable region FR3
GVPSRFSGSGSGTEFTLTISSLQPEDFATYYC

SEQ ID NO: 165 - protein, 32 aa, Artificial sequence
  Light chain variable region FR3
GIPDRFSGSGSGTDFTLTISRLEPEDFAVYYC

SEQ ID NO: 166 - protein, 32 aa, Artificial sequence
  Light chain variable region FR3
GIPARFSGSGSGTDFTLTISSLQAEDVAVYYC

SEQ ID NO: 167 - protein, 32 aa, Artificial sequence
  Light chain variable region FR3
GIPARFSGSGSGTEFTLTISSLQSEDFAFYFC

SEQ ID NO: 168 - protein, 32 aa, Artificial sequence
  Light chain variable region FR3
GIPARFSGSGSGTESTLTISSLQSEDCAVYYC

SEQ ID NO: 169 - protein, 8 aa, Artificial sequence
  Light chain variable region CDR3
QQRTNWYT

SEQ ID NO: 170 - protein, 10 aa, Artificial sequence
  Light chain variable region CDR3
QQYDSYSPIT

SEQ ID NO: 171 - protein, 9 aa, Artificial sequence
  Light chain variable region CDR3
QKCNSAPRT

SEQ ID NO: 172 - protein, 10 aa, Artificial sequence
  Light chain variable region CDR3
QQSFSTPPIT

SEQ ID NO: 173 - protein, 10 aa, Artificial sequence
  Light chain variable region CDR3
QQSYSIPPIT

SEQ ID NO: 174 - protein, 9 aa, Artificial sequence
  Light chain variable region CDR3
QKFNSAPLT

SEQ ID NO: 175 - protein, 9 aa, Artificial sequence
  Light chain variable region CDR3
QQYDSYSIT

SEQ ID NO: 176 - protein, 10 aa, Artificial sequence
  Light chain variable region CDR3
QQYDNWPPIT

SEQ ID NO: 177 - protein, 10 aa, Artificial sequence
  Light chain variable region CDR3
QQYSSYSPIT

SEQ ID NO: 178 - protein, 10 aa, Artificial sequence
  Light chain variable region CDR3
QQYNNWPPIT

SEQ ID NO: 179 - protein, 10 aa, Artificial sequence
  Light chain variable region CDR3
QQSYSTPPIT

SEQ ID NO: 180 - protein, 9 aa, Artificial sequence
  Light chain variable region CDR3
QQLNSYPYT

SEQ ID NO: 181 - protein, 9 aa, Artificial sequence
  Light chain variable region CDR3
QQYGSSPRT

SEQ ID NO: 182 - protein, 9 aa, Artificial sequence
  Light chain variable region CDR3
QQYYSTPYT

SEQ ID NO: 183 - protein, 9 aa, Artificial sequence
  Light chain variable region CDR3
QQVKIYPLT

SEQ ID NO: 184 - protein, 9 aa, Artificial sequence
  Light chain variable region CDR3
QQYENWPLT

SEQ ID NO: 185 - protein, 9 aa, Artificial sequence
  Light chain variable region CDR3
QQYNNWPST

SEQ ID NO: 186 - protein, 10 aa, Artificial sequence
  Light chain variable region FR4
FGQGTKLEIK

SEQ ID NO: 187 - protein, 10 aa, Artificial sequence
  Light chain variable region FR4
FGQGTRLEIK

SEQ ID NO: 188 - protein, 10 aa, Artificial sequence
  Light chain variable region FR4
FGQGTKVEIK

SEQ ID NO: 189 - protein, 10 aa, Artificial sequence
  Light chain variable region FR4
FGGGTKVEIK

SEQ ID NO: 190 - protein, 10 aa, Artificial sequence
  Light chain variable region FR4
FGQGSRLEIK

SEQ ID NO: 191 - protein, 10 aa, Artificial sequence
  Light chain variable region FR4
FGPGTKLEVT

SEQ ID NO: 192 - protein, 120 aa, Artificial sequence
  Heavy chain variable region
QVQLQESGPGLVKPSGTLSLTCAVSGGSISSSNWWSWVRQPPGKGLEWIGEIFHSGTTYYNPSLKSRVTILVDKSKNQFSLKLSSVTAADTAVYYCARDNTKSWDHFDHWGQGTLVTVSS

SEQ ID NO: 193 - protein, 119 aa, Artificial sequence
  Heavy chain variable region
QVQLQESGPGLVKPSGTLSLTCAVSGDSISSHNWWSWVRQPPGKGLEWIGEIYHSGITSYNPSLKSRVTISVDKSKNQFSLKLNSVTAADTAMYYCARGSGVISYFDYWGQGTLVTVSS

SEQ ID NO: 194 - protein, 121 aa, Artificial sequence
  Heavy chain variable region
QVELVESGGGVVQPGRSLRLSCGASGFTFSSYNMYWVRQAPGKGLEWVAGIWDDGNNKYYANSVKGRFTISRDNSKNTLYLQMNSLRTEDTALYYCAKDGWGSYGEYFQHWGQGTLVTVSS

SEQ ID NO: 195 - protein, 121 aa, Artificial sequence
  Heavy chain variable region
QVNLVESGGGVVQPGRSLKLSCAASGFTFSSYGMHWVRQAPGKGLEWVALIWSDGTNRYYTESVKGRFTISRDNSKNTLSLQMKSLRAEDTAVYYCAKDGWGTYGEYFQHWGQGTLVTVSS

SEQ ID NO: 196 - protein, 121 aa, Artificial sequence
  Heavy chain variable region
QVQLVESGGGVVQPGRSLRVSCIASGFFFSSYGMHWVRQAPGKGLEWVAVIWYDGSNEDYVDSVKGRFTISRDNSKNTLYLQMNSLRGEDTAMYYCARGGYNSGWWAFDIWGQGTMVTVSS

SEQ ID NO: 197 - protein, 118 aa, Artificial sequence
  Heavy chain variable region
QVQLQESGPRLVKPSETLSLTCAVSGYSISSGYYWGWIRQSPGMGLEWIAYIYHDGSTYCNPSLKSRVTMSVDTSKNQFSLKLRSVTAADTAVYYCARDGAAAPFDYWGQGTLVTVSS

SEQ ID NO: 198 - protein, 120 aa, Artificial sequence
  Heavy chain variable region
QVQLVESGGGVVQPGRSLRLSCAASGFTFSSFGMQWVRQGPGKGLEWVAVMWFDGSNKYYVDSVKGRFTISRDNSKNTLYLQMNSLRAEDTAVYYCARLDFSGWPLIDYWGQGTLVTVSS

SEQ ID NO: 199 - protein, 119 aa, Artificial sequence
  Heavy chain variable region
QVQLQESGPGLVKPSGTLSLTCAVSGDSISSNNWWSWVRQPPGKGLEWIGEIYPGGNPNYNPSLKSRVTISVDKSKNQFSLKLNSVTAADTAVYYCARGSGVISYFDYWGQGTLVTVSS

SEQ ID NO: 200 - protein, 121 aa, Artificial sequence
  Heavy chain variable region
QVQLVESGGGVVQPGRSLRVSCAASGFIFSTYGMHWVRQAPGKGLEWVAVIWYDGSNEDYVDSVKGRFTISRDNSKNTLYLQMNSLRGEDTAVYYCARGGYNSGWWAFDVWGQGTLVTVSS

SEQ ID NO: 201 - protein, 120 aa, Artificial sequence
  Heavy chain variable region
QVQLVESGGGVVQPGRSLRLSCAASGFTFSSFGMQWVRQGPGKGLEWVAIMWFDGSNKYYVDSVKGRFTISRDNSKNTLYLQMNSLRAEDTAVYYCARLDFSGWPLIDYWGQGTLVTVSS

SEQ ID NO: 202 - protein, 121 aa, Artificial sequence
  Heavy chain variable region
QVNLVESGGGVVQPGRSLKLSCAASGFTFSSYGMHWVRQAPGKGLEWVAFIWSDGTNRYYPESVKGRFTISRDDSRNTVSLQMNSLRPEDTAVYYCARDGWGTYGEYFQHWGQGTLVTVSS

SEQ ID NO: 203 - protein, 123 aa, Artificial sequence
  Heavy chain variable region
QVQLVESGGGVVQPEKSLRLSCAASGFTFSHYGMHWVRQVPGKGLEWVAVIWYDGIKRYYVESVKGRFTISRDNSKNTLYLQMNRLRAEDTAVYYCARDGGFGESNYYGLDVWGQGTTVTVSS

SEQ ID NO: 204 - protein, 123 aa, Artificial sequence
  Heavy chain variable region
QVQLVESGGGVVQPGRSLRLSCAASGFTFSHYGMHWVRQAPGKGLEWVAVIWYDGIKKDYVESVKGRFTISRDNSKNTLYLQMNRLRAEDTAVYYCARDGGFGELNYYGLDVWGQGTTVTVSS

SEQ ID NO: 205 - protein, 123 aa, Artificial sequence
  Heavy chain variable region
QVQLVESGGAVVQPGRSLRLSCAASGFTFSHYGMHWVRQAPGKGLEWVAVIWYDGIKSYYVESVKGRFTISRDNSKNTLYLQMDRLRAEDTAVYYCARDGGFGESNYYGLDVWGQGTTVTVSS

SEQ ID NO: 206 - protein, 116 aa, Artificial sequence
  Heavy chain variable region
QVQLQESGPGLVKPSGTLSLTCAVSGGSISSSNWWSWVRQPPGKGLEWIGEIYHDGSTDYNPSLKSRVIISVDKSKNQFSLKVRSVTAADTAVYYCARDNWGFDYWGQGTLVTVSS

SEQ ID NO: 207 - protein, 123 aa, Artificial sequence
  Heavy chain variable region
QVQLVESGGGVVQPGRSLRLSCEASGFTFSHYGMHWVRQAPGKGLEWVAVIWYDGIKKYYIESVKGRFIISRDNSKNTLYLQMNRLRAEDTAVYYCARDGGFGELNYYGLDVWGQGTTVTVSS

SEQ ID NO: 208 - protein, 123 aa, Artificial sequence
  Heavy chain variable region
QVQLVQSGGGVVQPGRSLRLSCAASGFTFSHYGMHWVRQAPGKGLEWVAVIWYDGIKKYYVESVKGRFTISRDNSKNTLYLQMNRLRAEDTAVYYCARDGGFGELNYYGLDVWGQGTTVTVSS

SEQ ID NO: 209 - protein, 123 aa, Artificial sequence
  Heavy chain variable region
QVQLVESGGGVVQPGRSLRLSCEGSGFTFSHYGMHWVRQAPGKGLEWVAVIWYDGIKKNYVDSLKGRFTISRDNSKNTLYLQMNSLRAEDTAVYYCARDGGFGELNYYGMDVWGQGTTVTVSS

SEQ ID NO: 210 - protein, 123 aa, Artificial sequence
  Heavy chain variable region
QVQLVESGGGVVQPGRSLRLSCVASGFTFSHYGMHWVRQAPGKGLEWVAVIWYDGIKKYYVESVKGRFTISRDNSKNTLNLQMNRLRAEDTAVYYCARDGGFGESNYYGLDVWGQGTTVTVSS

SEQ ID NO: 211 - protein, 123 aa, Artificial sequence
  Heavy chain variable region
QVQLVESGGGVVQPGRSLRLSCEASGFTFSHYGMHWVRQAPGKGLEWVAVIWYDGIKTNYVESVKGRFTISRDNSKNTLNLQMNRLRAEDTAVYYCARDGGFGESNYYGLDVWGQGTTVTVSS

SEQ ID NO: 212 - protein, 123 aa, Artificial sequence
  Heavy chain variable region
QVQLVESGGGVVQPGRSLRLSCEASGFTFSHYGMHWVRQAPGKGLEWVAVIWYDGIMKNYIESVKGRFTISRDNSKNTLYLQMNRLRAEDTAVYYCARDGGFGELNYYGLDVWGQGTTVTVSS

SEQ ID NO: 213 - protein, 122 aa, Artificial sequence
  Heavy chain variable region
QVQLVESGGGVVQPGTSLRLSCVASGFTFSNDGMHWVRQAPGMGLEWVAIMWFDGGSKYYADSVKGRFTISRDNSKNTLYLQMNNLRAEDTAVYYCARDHPHYLGSGSFDYWGQGTLVTVSS

SEQ ID NO: 214 - protein, 123 aa, Artificial sequence
  Heavy chain variable region
QVQLVESGGDVVQPGRSLRLSCEASGFTFSHYGMHWVRQAPGKGLEWVAVVWYDGIKKYYVESVKGRFTISRDNSKNTLYLQMNRLRAEDTAVYYCARDGGFGELNYYGLDVWGQGTTVTVSS

SEQ ID NO: 215 - protein, 119 aa, Artificial sequence
  Heavy chain variable region
QVQLQQSGPGLVKPSQTLSLTCAISGDSVSSTSAVWNWIRQSPSRGLEWLGRTCYRSKWYNDYAVSVKSRITITPDTSKNQFSLRLNPVTPEDTAVYYCARGDFRFDSWGQGTLVTVSS

SEQ ID NO: 216 - protein, 123 aa, Artificial sequence
  Heavy chain variable region
QVQLVESGGGVVQPGRSLRLSCEASGFTFSHYGMHWVRQAPGKGLEWVAVIWYDGIKTYYVESVKGRFTISRDNSKNTLNLQMNRLRAEDTAVYYCARDGGFGESNYYGLDVWGQGTTVTVSS

SEQ ID NO: 217 - protein, 118 aa, Artificial sequence
  Heavy chain variable region
QVQLQESGPGLVKPSETLSLTCAVSGYSISSGYFWAWIRQPPGKGLEWIGSIYHSGRTHYNPSLKSRVIISLDTSKNQFSLKLRSVTAADSAVYYCAREGYASGSYYWGQGTLVTVSS

SEQ ID NO: 218 - protein, 121 aa, Artificial sequence
  Heavy chain variable region
QVQLVESGGGVVQPGRSLRLSCATSGFIFSSYGMHWVRQAPGKGLDWVAVIWYDGSNKYYADSVKGRFTISRDNSKNTLYLQMNSLRVEDTAVYYCARETSSWYVGYLQHWGQGTLVTVSS

SEQ ID NO: 219 - protein, 118 aa, Artificial sequence
  Heavy chain variable region
QVQLQESGPGLVKPSETLSLTCAVSGYSINSGYFWAWIRQPPGMGLEWIGSIYHSGRTHYNPSLKSRVIISLDTSKNQFSLKLRSVTAADSAVYYCAREGYASGSYYWGQGTLVTVSS

SEQ ID NO: 220 - protein, 123 aa, Artificial sequence
  Heavy chain variable region
QVQLVESGGGVVQPGRSLRLSCAASGFTFSHYGMHWVRQAPGKGLEWVAVIWYDGIKKNYVESVKGRFTISRDNSKNTLNLQMNRLRAEDTAVYYCARDGGFGESNYYGLDVWGQGTTVTVSS

SEQ ID NO: 221 - protein, 106 aa, Artificial sequence
  Light chain variable region
EIVLTQSPATLSLSPGERATLSCRASQSVGSYLAWYQQKPGQAPSLLIYDASNRATGIPARFSGSGSGTDFTLTISSLEPEDFAVYYCQQRTNWYTFGQGTKLEIK

SEQ ID NO: 222 - protein, 108 aa, Artificial sequence
  Light chain variable region
DIQMTQSPSTLSASVGDRVTITCRASQSIGNWLAWYQQKPGKAPKLLIYKASSLESGVPSRFSGSGSGTEFTLTISSLQPDDFATYYCQQYDSYSPITFGQGTRLEIK

SEQ ID NO: 223 - protein, 107 aa, Artificial sequence
  Light chain variable region
DIQMTQSPSSLSASLGDRVTITCRATQGISNYLAWYQQKPGKVPNLLIYAASTLQSGVPSRFSGSGSGTDLTLTISSLQPEDVATYYCQKCNSAPRTFGQGTKVEIK

SEQ ID NO: 224 - protein, 108 aa, Artificial sequence
  Light chain variable region
DIQMTQSPSSLSASVGERVTITCRASQNINSYLSWYQQKPGKAPKLLIYAASSLQNGVPSRFSGSGSGTDFTLTISSLQPEDFATYYCQQSFSTPPITFGQGTRLEIK

SEQ ID NO: 225 - protein, 108 aa, Artificial sequence
  Light chain variable region
DIQMTQSPSSLSASVGDRVTITCRASQNINSYLHWYQQKPGKAPKLLIYAASSLQSGVPSRFSGSGSGTDFTLTISSLQPEDFAIYYCQQSYSIPPITFGQGTRLEIK

SEQ ID NO: 226 - protein, 107 aa, Artificial sequence
  Light chain variable region
DIQMTQSPSSLSASVGDRVTITCRASQGISHFLAWYQQKPGKVPKLLIYAASTLQSGVPSRFSGSGSGTDFTLTISSLQPEDVATYYCQKFNSAPLTFGGGTKVEIK

SEQ ID NO: 227 - protein, 107 aa, Artificial sequence
  Light chain variable region
DIQMTQSPSTLSASVGDRVTITCRASQSISNWLAWYQQKPGKAPKVLIYKASSLESGVPSRFSGSGSGTEFTLTINSLQPDDFATYYCQQYDSYSITFGQGTRLEIK

SEQ ID NO: 228 - protein, 108 aa, Artificial sequence
  Light chain variable region
QVVMTQSPATLSVSPGERATLSCRASQSVSSKLAWYQQKPGQAPRLIIYGASTRATGIPARFSGSGSGTEFTLTISSLQSEDFAVYYCQQYDNWPPITFGQGTRLEIK

SEQ ID NO: 229 - protein, 108 aa, Artificial sequence
  Light chain variable region
DIQMTQSPSTLSASVGDRVTITCRASQSIGHWLAWYQQKPGKAPKLLIYKASSLESGVPSRFRGSGSGTEFTLTISSLQPDDFATYYCQQYSSYSPITFGQGSRLEIK

SEQ ID NO: 230 - protein, 108 aa, Artificial sequence
  Light chain variable region
EIVMTQSPATLSVSPGERATLSCRASQSVSSNLAWYQQKPGQAPRLLIYGASTRATGIPARFSGSGSGTEFTLTISSLQSEDFAVYYCQQYNNWPPITFGQGTRLEIK

SEQ ID NO: 231 - protein, 108 aa, Artificial sequence
  Light chain variable region
DIQMTQSPSSLSASVGDRVTITCRASQSINSYLHWYQQKPGKAPKLLIYAASSLQSGVPSRFSGSGSGTDFTLTISSLQPEDFATYYCQQSYSTPPITFGQGTRLEIK

SEQ ID NO: 232 - protein, 107 aa, Artificial sequence
  Light chain variable region
DIQLTQSPSFLSASVGDRVTITCRASQGINSYLGWYQRKPGKAPKLLIYIASTLQSGVPSRFSGSGSGTEFTLTISSLQPEDFATYYCQQLNSYPYTFGQGTKLEIK

SEQ ID NO: 233 - protein, 107 aa, Artificial sequence
  Light chain variable region
DIQLTQSPSFLSASVGDRVTITCRASQGISSYLGWYQQKPGKAPKLLIYVASTLQSGVPSRFSGSGSGTEFTLTISSLQPEDFATYYCQQLNSYPYTFGQGTKLEIK

SEQ ID NO: 234 - protein, 108 aa, Artificial sequence
  Light chain variable region
EIVLTQFPGTLSLSPGERATLSCRSSQSVSSSYLAWYQQKPGQAPRLLISGASSRATGIPDRFSGSGSGTDFTLTISRLEPEDFAVYYCQQYGSSPRTFGQGTKVEIK

SEQ ID NO: 235 - protein, 107 aa, Artificial sequence
  Light chain variable region
DIQLTQSPSFLSASVGDRVTITCRASQGISSYLGWYQQKPGKAPKLLIYIASTLQSGVPSRFSGSGSGTEFTLTISSLQPEDFATYYCQQLNSYPYTFGQGTKLEIK

SEQ ID NO: 236 - protein, 107 aa, Artificial sequence
  Light chain variable region
EIVLTQSPATLSLSPGERATLSCRASQSVSSYLAWYQQKPGQAPRLLIYDASNRATGIPARFSGSGSGTDFTLTISSLQAEDVAVYYCQQYYSTPYTFGQGTKLEIK

SEQ ID NO: 237 - protein, 107 aa, Artificial sequence
  Light chain variable region
DIQLTQSPSFLSASVGDRVTITCRASQGISSYLAWYQQKPGKAPKLLIYAASTLQSGVPSRFSGSGSGTEFTLTISSLQPEDFATYYCQQVKIYPLTFGGGTKVEIK

SEQ ID NO: 238 - protein, 107 aa, Artificial sequence
  Light chain variable region
EIVMTQSPATLSVSPGERATLSCRSSQSVNNYLAWFQQKPGQAPRLLIYDSSTRATGIPARFSGSGSGTEFTLTISSLQSEDFAFYFCQQYENWPLTFGGGTKVEIK

SEQ ID NO: 239 - protein, 107 aa, Artificial sequence
  Light chain variable region
EIVMTQSPATLSVSPGERVSLSCRASQSVNGNVAWYQQKPGQAPRLLIYAASTRATGIPARFSGSGSGTESTLTISSLQSEDCAVYYCQQYNNWPSTFGPGTKLEVT

SEQ ID NO: 240 - protein, 107 aa, Artificial sequence
  Light chain variable region
EIVMTQSPATLSVSPGERATLSCRSSQSVNSYLAWFQQKPGQAPRLLIYDSSTRATGIPARFSGSGSGTEFTLTISSLQSEDFAFYFCQQYENWPLTFGGGTKVEIK

SEQ ID NO: 241 - protein, 450 aa, Artificial sequence
  Heavy chain
QVQLQESGPGLVKPSGTLSLTCAVSGGSISSSNWWSWVRQPPGKGLEWIGEIFHSGTTYYNPSLKSRVTILVDKSKNQFSLKLSSVTAADTAVYYCARDNTKSWDHFDHWGQGTLVTVSSASTKGPSVFPLAPSSKSTSGGTAALGCLVKDYFPEPVTVSWNSGALTSGVHTFPAVLQSSGLYSLSSVVTVPSSSLGTQTYICNVNHKPSNTKVDKKVEPKSCDKTHTCPPCPAPELLGGPSVFLFPPKPKDTLMISRTPEVTCVVVDVSHEDPEVKFNWYVDGVEVHNAKTKPREEQYNSTYRVVSVLTVLHQDWLNGKEYKCKVSNKALPAPIEKTISKAKGQPREPQVYTLPPSREEMTKNQVSLTCLVKGFYPSDIAVEWESNGQPENNYKTTPPVLDSDGSFFLYSKLTVDKSRWQQGNVFSCSVMHEALHNHYTQKSLSLSPGK

SEQ ID NO: 242 - protein, 449 aa, Artificial sequence
  Heavy chain
QVQLQESGPGLVKPSGTLSLTCAVSGDSISSHNWWSWVRQPPGKGLEWIGEIYHSGITSYNPSLKSRVTISVDKSKNQFSLKLNSVTAADTAMYYCARGSGVISYFDYWGQGTLVTVSSASTKGPSVFPLAPSSKSTSGGTAALGCLVKDYFPEPVTVSWNSGALTSGVHTFPAVLQSSGLYSLSSVVTVPSSSLGTQTYICNVNHKPSNTKVDKKVEPKSCDKTHTCPPCPAPELLGGPSVFLFPPKPKDTLMISRTPEVTCVVVDVSHEDPEVKFNWYVDGVEVHNAKTKPREEQYNSTYRVVSVLTVLHQDWLNGKEYKCKVSNKALPAPIEKTISKAKGQPREPQVYTLPPSREEMTKNQVSLTCLVKGFYPSDIAVEWESNGQPENNYKTTPPVLDSDGSFFLYSKLTVDKSRWQQGNVFSCSVMHEALHNHYTQKSLSLSPGK

SEQ ID NO: 243 - protein, 451 aa, Artificial sequence
  Heavy chain
QVELVESGGGVVQPGRSLRLSCGASGFTFSSYNMYWVRQAPGKGLEWVAGIWDDGNNKYYANSVKGRFTISRDNSKNTLYLQMNSLRTEDTALYYCAKDGWGSYGEYFQHWGQGTLVTVSSASTKGPSVFPLAPSSKSTSGGTAALGCLVKDYFPEPVTVSWNSGALTSGVHTFPAVLQSSGLYSLSSVVTVPSSSLGTQTYICNVNHKPSNTKVDKKVEPKSCDKTHTCPPCPAPELLGGPSVFLFPPKPKDTLMISRTPEVTCVVVDVSHEDPEVKFNWYVDGVEVHNAKTKPREEQYNSTYRVVSVLTVLHQDWLNGKEYKCKVSNKALPAPIEKTISKAKGQPREPQVYTLPPSREEMTKNQVSLTCLVKGFYPSDIAVEWESNGQPENNYKTTPPVLDSDGSFFLYSKLTVDKSRWQQGNVFSCSVMHEALHNHYTQKSLSLSPGK

SEQ ID NO: 244 - protein, 451 aa, Artificial sequence
  Heavy chain
QVNLVESGGGVVQPGRSLKLSCAASGFTFSSYGMHWVRQAPGKGLEWVALIWSDGTNRYYTESVKGRFTISRDNSKNTLSLQMKSLRAEDTAVYYCAKDGWGTYGEYFQHWGQGTLVTVSSASTKGPSVFPLAPSSKSTSGGTAALGCLVKDYFPEPVTVSWNSGALTSGVHTFPAVLQSSGLYSLSSVVTVPSSSLGTQTYICNVNHKPSNTKVDKKVEPKSCDKTHTCPPCPAPELLGGPSVFLFPPKPKDTLMISRTPEVTCVVVDVSHEDPEVKFNWYVDGVEVHNAKTKPREEQYNSTYRVVSVLTVLHQDWLNGKEYKCKVSNKALPAPIEKTISKAKGQPREPQVYTLPPSREEMTKNQVSLTCLVKGFYPSDIAVEWESNGQPENNYKTTPPVLDSDGSFFLYSKLTVDKSRWQQGNVFSCSVMHEALHNHYTQKSLSLSPGK

SEQ ID NO: 245 - protein, 451 aa, Artificial sequence
  Heavy chain
QVQLVESGGGVVQPGRSLRVSCIASGFFFSSYGMHWVRQAPGKGLEWVAVIWYDGSNEDYVDSVKGRFTISRDNSKNTLYLQMNSLRGEDTAMYYCARGGYNSGWWAFDIWGQGTMVTVSSASTKGPSVFPLAPSSKSTSGGTAALGCLVKDYFPEPVTVSWNSGALTSGVHTFPAVLQSSGLYSLSSVVTVPSSSLGTQTYICNVNHKPSNTKVDKKVEPKSCDKTHTCPPCPAPELLGGPSVFLFPPKPKDTLMISRTPEVTCVVVDVSHEDPEVKFNWYVDGVEVHNAKTKPREEQYNSTYRVVSVLTVLHQDWLNGKEYKCKVSNKALPAPIEKTISKAKGQPREPQVYTLPPSREEMTKNQVSLTCLVKGFYPSDIAVEWESNGQPENNYKTTPPVLDSDGSFFLYSKLTVDKSRWQQGNVFSCSVMHEALHNHYTQKSLSLSPGK

SEQ ID NO: 246 - protein, 448 aa, Artificial sequence
  Heavy chain
QVQLQESGPRLVKPSETLSLTCAVSGYSISSGYYWGWIRQSPGMGLEWIAYIYHDGSTYCNPSLKSRVTMSVDTSKNQFSLKLRSVTAADTAVYYCARDGAAAPFDYWGQGTLVTVSSASTKGPSVFPLAPSSKSTSGGTAALGCLVKDYFPEPVTVSWNSGALTSGVHTFPAVLQSSGLYSLSSVVTVPSSSLGTQTYICNVNHKPSNTKVDKKVEPKSCDKTHTCPPCPAPELLGGPSVFLFPPKPKDTLMISRTPEVTCVVVDVSHEDPEVKFNWYVDGVEVHNAKTKPREEQYNSTYRVVSVLTVLHQDWLNGKEYKCKVSNKALPAPIEKTISKAKGQPREPQVYTLPPSREEMTKNQVSLTCLVKGFYPSDIAVEWESNGQPENNYKTTPPVLDSDGSFFLYSKLTVDKSRWQQGNVFSCSVMHEALHNHYTQKSLSLSPGK

SEQ ID NO: 247 - protein, 450 aa, Artificial sequence
  Heavy chain
QVQLVESGGGVVQPGRSLRLSCAASGFTFSSFGMQWVRQGPGKGLEWVAVMWFDGSNKYYVDSVKGRFTISRDNSKNTLYLQMNSLRAEDTAVYYCARLDFSGWPLIDYWGQGTLVTVSSASTKGPSVFPLAPSSKSTSGGTAALGCLVKDYFPEPVTVSWNSGALTSGVHTFPAVLQSSGLYSLSSVVTVPSSSLGTQTYICNVNHKPSNTKVDKKVEPKSCDKTHTCPPCPAPELLGGPSVFLFPPKPKDTLMISRTPEVTCVVVDVSHEDPEVKFNWYVDGVEVHNAKTKPREEQYNSTYRVVSVLTVLHQDWLNGKEYKCKVSNKALPAPIEKTISKAKGQPREPQVYTLPPSREEMTKNQVSLTCLVKGFYPSDIAVEWESNGQPENNYKTTPPVLDSDGSFFLYSKLTVDKSRWQQGNVFSCSVMHEALHNHYTQKSLSLSPGK

SEQ ID NO: 248 - protein, 449 aa, Artificial sequence
  Heavy chain
QVQLQESGPGLVKPSGTLSLTCAVSGDSISSNNWWSWVRQPPGKGLEWIGEIYPGGNPNYNPSLKSRVTISVDKSKNQFSLKLNSVTAADTAVYYCARGSGVISYFDYWGQGTLVTVSSASTKGPSVFPLAPSSKSTSGGTAALGCLVKDYFPEPVTVSWNSGALTSGVHTFPAVLQSSGLYSLSSVVTVPSSSLGTQTYICNVNHKPSNTKVDKKVEPKSCDKTHTCPPCPAPELLGGPSVFLFPPKPKDTLMISRTPEVTCVVVDVSHEDPEVKFNWYVDGVEVHNAKTKPREEQYNSTYRVVSVLTVLHQDWLNGKEYKCKVSNKALPAPIEKTISKAKGQPREPQVYTLPPSREEMTKNQVSLTCLVKGFYPSDIAVEWESNGQPENNYKTTPPVLDSDGSFFLYSKLTVDKSRWQQGNVFSCSVMHEALHNHYTQKSLSLSPGK

SEQ ID NO: 249 - protein, 451 aa, Artificial sequence
  Heavy chain
QVQLVESGGGVVQPGRSLRVSCAASGFIFSTYGMHWVRQAPGKGLEWVAVIWYDGSNEDYVDSVKGRFTISRDNSKNTLYLQMNSLRGEDTAVYYCARGGYNSGWWAFDVWGQGTLVTVSSASTKGPSVFPLAPSSKSTSGGTAALGCLVKDYFPEPVTVSWNSGALTSGVHTFPAVLQSSGLYSLSSVVTVPSSSLGTQTYICNVNHKPSNTKVDKKVEPKSCDKTHTCPPCPAPELLGGPSVFLFPPKPKDTLMISRTPEVTCVVVDVSHEDPEVKFNWYVDGVEVHNAKTKPREEQYNSTYRVVSVLTVLHQDWLNGKEYKCKVSNKALPAPIEKTISKAKGQPREPQVYTLPPSREEMTKNQVSLTCLVKGFYPSDIAVEWESNGQPENNYKTTPPVLDSDGSFFLYSKLTVDKSRWQQGNVFSCSVMHEALHNHYTQKSLSLSPGK

SEQ ID NO: 250 - protein, 450 aa, Artificial sequence
  Heavy chain
QVQLVESGGGVVQPGRSLRLSCAASGFTFSSFGMQWVRQGPGKGLEWVAIMWFDGSNKYYVDSVKGRFTISRDNSKNTLYLQMNSLRAEDTAVYYCARLDFSGWPLIDYWGQGTLVTVSSASTKGPSVFPLAPSSKSTSGGTAALGCLVKDYFPEPVTVSWNSGALTSGVHTFPAVLQSSGLYSLSSVVTVPSSSLGTQTYICNVNHKPSNTKVDKKVEPKSCDKTHTCPPCPAPELLGGPSVFLFPPKPKDTLMISRTPEVTCVVVDVSHEDPEVKFNWYVDGVEVHNAKTKPREEQYNSTYRVVSVLTVLHQDWLNGKEYKCKVSNKALPAPIEKTISKAKGQPREPQVYTLPPSREEMTKNQVSLTCLVKGFYPSDIAVEWESNGQPENNYKTTPPVLDSDGSFFLYSKLTVDKSRWQQGNVFSCSVMHEALHNHYTQKSLSLSPGK

SEQ ID NO: 251 - protein, 451 aa, Artificial sequence
  Heavy chain
QVNLVESGGGVVQPGRSLKLSCAASGFTFSSYGMHWVRQAPGKGLEWVAFIWSDGTNRYYPESVKGRFTISRDDSRNTVSLQMNSLRPEDTAVYYCARDGWGTYGEYFQHWGQGTLVTVSSASTKGPSVFPLAPSSKSTSGGTAALGCLVKDYFPEPVTVSWNSGALTSGVHTFPAVLQSSGLYSLSSVVTVPSSSLGTQTYICNVNHKPSNTKVDKKVEPKSCDKTHTCPPCPAPELLGGPSVFLFPPKPKDTLMISRTPEVTCVVVDVSHEDPEVKFNWYVDGVEVHNAKTKPREEQYNSTYRVVSVLTVLHQDWLNGKEYKCKVSNKALPAPIEKTISKAKGQPREPQVYTLPPSREEMTKNQVSLTCLVKGFYPSDIAVEWESNGQPENNYKTTPPVLDSDGSFFLYSKLTVDKSRWQQGNVFSCSVMHEALHNHYTQKSLSLSPGK

SEQ ID NO: 252 - protein, 453 aa, Artificial sequence
  Heavy chain
QVQLVESGGGVVQPEKSLRLSCAASGFTFSHYGMHWVRQVPGKGLEWVAVIWYDGIKRYYVESVKGRFTISRDNSKNTLYLQMNRLRAEDTAVYYCARDGGFGESNYYGLDVWGQGTTVTVSSASTKGPSVFPLAPSSKSTSGGTAALGCLVKDYFPEPVTVSWNSGALTSGVHTFPAVLQSSGLYSLSSVVTVPSSSLGTQTYICNVNHKPSNTKVDKKVEPKSCDKTHTCPPCPAPELLGGPSVFLFPPKPKDTLMISRTPEVTCVVVDVSHEDPEVKFNWYVDGVEVHNAKTKPREEQYNSTYRVVSVLTVLHQDWLNGKEYKCKVSNKALPAPIEKTISKAKGQPREPQVYTLPPSREEMTKNQVSLTCLVKGFYPSDIAVEWESNGQPENNYKTTPPVLDSDGSFFLYSKLTVDKSRWQQGNVFSCSVMHEALHNHYTQKSLSLSPGK

SEQ ID NO: 253 - protein, 453 aa, Artificial sequence
  Heavy chain
QVQLVESGGGVVQPGRSLRLSCAASGFTFSHYGMHWVRQAPGKGLEWVAVIWYDGIKKDYVESVKGRFTISRDNSKNTLYLQMNRLRAEDTAVYYCARDGGFGELNYYGLDVWGQGTTVTVSSASTKGPSVFPLAPSSKSTSGGTAALGCLVKDYFPEPVTVSWNSGALTSGVHTFPAVLQSSGLYSLSSVVTVPSSSLGTQTYICNVNHKPSNTKVDKKVEPKSCDKTHTCPPCPAPELLGGPSVFLFPPKPKDTLMISRTPEVTCVVVDVSHEDPEVKFNWYVDGVEVHNAKTKPREEQYNSTYRVVSVLTVLHQDWLNGKEYKCKVSNKALPAPIEKTISKAKGQPREPQVYTLPPSREEMTKNQVSLTCLVKGFYPSDIAVEWESNGQPENNYKTTPPVLDSDGSFFLYSKLTVDKSRWQQGNVFSCSVMHEALHNHYTQKSLSLSPGK

SEQ ID NO: 254 - protein, 453 aa, Artificial sequence
  Heavy chain
QVQLVESGGAVVQPGRSLRLSCAASGFTFSHYGMHWVRQAPGKGLEWVAVIWYDGIKSYYVESVKGRFTISRDNSKNTLYLQMDRLRAEDTAVYYCARDGGFGESNYYGLDVWGQGTTVTVSSASTKGPSVFPLAPSSKSTSGGTAALGCLVKDYFPEPVTVSWNSGALTSGVHTFPAVLQSSGLYSLSSVVTVPSSSLGTQTYICNVNHKPSNTKVDKKVEPKSCDKTHTCPPCPAPELLGGPSVFLFPPKPKDTLMISRTPEVTCVVVDVSHEDPEVKFNWYVDGVEVHNAKTKPREEQYNSTYRVVSVLTVLHQDWLNGKEYKCKVSNKALPAPIEKTISKAKGQPREPQVYTLPPSREEMTKNQVSLTCLVKGFYPSDIAVEWESNGQPENNYKTTPPVLDSDGSFFLYSKLTVDKSRWQQGNVFSCSVMHEALHNHYTQKSLSLSPGK

SEQ ID NO: 255 - protein, 446 aa, Artificial sequence
  Heavy chain
QVQLQESGPGLVKPSGTLSLTCAVSGGSISSSNWWSWVRQPPGKGLEWIGEIYHDGSTDYNPSLKSRVIISVDKSKNQFSLKVRSVTAADTAVYYCARDNWGFDYWGQGTLVTVSSASTKGPSVFPLAPSSKSTSGGTAALGCLVKDYFPEPVTVSWNSGALTSGVHTFPAVLQSSGLYSLSSVVTVPSSSLGTQTYICNVNHKPSNTKVDKKVEPKSCDKTHTCPPCPAPELLGGPSVFLFPPKPKDTLMISRTPEVTCVVVDVSHEDPEVKFNWYVDGVEVHNAKTKPREEQYNSTYRVVSVLTVLHQDWLNGKEYKCKVSNKALPAPIEKTISKAKGQPREPQVYTLPPSREEMTKNQVSLTCLVKGFYPSDIAVEWESNGQPENNYKTTPPVLDSDGSFFLYSKLTVDKSRWQQGNVFSCSVMHEALHNHYTQKSLSLSPGK

SEQ ID NO: 256 - protein, 453 aa, Artificial sequence
  Heavy chain
QVQLVESGGGVVQPGRSLRLSCEASGFTFSHYGMHWVRQAPGKGLEWVAVIWYDGIKKYYIESVKGRFIISRDNSKNTLYLQMNRLRAEDTAVYYCARDGGFGELNYYGLDVWGQGTTVTVSSASTKGPSVFPLAPSSKSTSGGTAALGCLVKDYFPEPVTVSWNSGALTSGVHTFPAVLQSSGLYSLSSVVTVPSSSLGTQTYICNVNHKPSNTKVDKKVEPKSCDKTHTCPPCPAPELLGGPSVFLFPPKPKDTLMISRTPEVTCVVVDVSHEDPEVKFNWYVDGVEVHNAKTKPREEQYNSTYRVVSVLTVLHQDWLNGKEYKCKVSNKALPAPIEKTISKAKGQPREPQVYTLPPSREEMTKNQVSLTCLVKGFYPSDIAVEWESNGQPENNYKTTPPVLDSDGSFFLYSKLTVDKSRWQQGNVFSCSVMHEALHNHYTQKSLSLSPGK

SEQ ID NO: 257 - protein, 453 aa, Artificial sequence
  Heavy chain
QVQLVQSGGGVVQPGRSLRLSCAASGFTFSHYGMHWVRQAPGKGLEWVAVIWYDGIKKYYVESVKGRFTISRDNSKNTLYLQMNRLRAEDTAVYYCARDGGFGELNYYGLDVWGQGTTVTVSSASTKGPSVFPLAPSSKSTSGGTAALGCLVKDYFPEPVTVSWNSGALTSGVHTFPAVLQSSGLYSLSSVVTVPSSSLGTQTYICNVNHKPSNTKVDKKVEPKSCDKTHTCPPCPAPELLGGPSVFLFPPKPKDTLMISRTPEVTCVVVDVSHEDPEVKFNWYVDGVEVHNAKTKPREEQYNSTYRVVSVLTVLHQDWLNGKEYKCKVSNKALPAPIEKTISKAKGQPREPQVYTLPPSREEMTKNQVSLTCLVKGFYPSDIAVEWESNGQPENNYKTTPPVLDSDGSFFLYSKLTVDKSRWQQGNVFSCSVMHEALHNHYTQKSLSLSPGK

SEQ ID NO: 258 - protein, 453 aa, Artificial sequence
  Heavy chain
QVQLVESGGGVVQPGRSLRLSCEGSGFTFSHYGMHWVRQAPGKGLEWVAVIWYDGIKKNYVDSLKGRFTISRDNSKNTLYLQMNSLRAEDTAVYYCARDGGFGELNYYGMDVWGQGTTVTVSSASTKGPSVFPLAPSSKSTSGGTAALGCLVKDYFPEPVTVSWNSGALTSGVHTFPAVLQSSGLYSLSSVVTVPSSSLGTQTYICNVNHKPSNTKVDKKVEPKSCDKTHTCPPCPAPELLGGPSVFLFPPKPKDTLMISRTPEVTCVVVDVSHEDPEVKFNWYVDGVEVHNAKTKPREEQYNSTYRVVSVLTVLHQDWLNGKEYKCKVSNKALPAPIEKTISKAKGQPREPQVYTLPPSREEMTKNQVSLTCLVKGFYPSDIAVEWESNGQPENNYKTTPPVLDSDGSFFLYSKLTVDKSRWQQGNVFSCSVMHEALHNHYTQKSLSLSPGK

SEQ ID NO: 259 - protein, 453 aa, Artificial sequence
  Heavy chain
QVQLVESGGGVVQPGRSLRLSCVASGFTFSHYGMHWVRQAPGKGLEWVAVIWYDGIKKYYVESVKGRFTISRDNSKNTLNLQMNRLRAEDTAVYYCARDGGFGESNYYGLDVWGQGTTVTVSSASTKGPSVFPLAPSSKSTSGGTAALGCLVKDYFPEPVTVSWNSGALTSGVHTFPAVLQSSGLYSLSSVVTVPSSSLGTQTYICNVNHKPSNTKVDKKVEPKSCDKTHTCPPCPAPELLGGPSVFLFPPKPKDTLMISRTPEVTCVVVDVSHEDPEVKFNWYVDGVEVHNAKTKPREEQYNSTYRVVSVLTVLHQDWLNGKEYKCKVSNKALPAPIEKTISKAKGQPREPQVYTLPPSREEMTKNQVSLTCLVKGFYPSDIAVEWESNGQPENNYKTTPPVLDSDGSFFLYSKLTVDKSRWQQGNVFSCSVMHEALHNHYTQKSLSLSPGK

SEQ ID NO: 260 - protein, 453 aa, Artificial sequence
  Heavy chain
QVQLVESGGGVVQPGRSLRLSCEASGFTFSHYGMHWVRQAPGKGLEWVAVIWYDGIKTNYVESVKGRFTISRDNSKNTLNLQMNRLRAEDTAVYYCARDGGFGESNYYGLDVWGQGTTVTVSSASTKGPSVFPLAPSSKSTSGGTAALGCLVKDYFPEPVTVSWNSGALTSGVHTFPAVLQSSGLYSLSSVVTVPSSSLGTQTYICNVNHKPSNTKVDKKVEPKSCDKTHTCPPCPAPELLGGPSVFLFPPKPKDTLMISRTPEVTCVVVDVSHEDPEVKFNWYVDGVEVHNAKTKPREEQYNSTYRVVSVLTVLHQDWLNGKEYKCKVSNKALPAPIEKTISKAKGQPREPQVYTLPPSREEMTKNQVSLTCLVKGFYPSDIAVEWESNGQPENNYKTTPPVLDSDGSFFLYSKLTVDKSRWQQGNVFSCSVMHEALHNHYTQKSLSLSPGK

SEQ ID NO: 261 - protein, 453 aa, Artificial sequence
  Heavy chain
QVQLVESGGGVVQPGRSLRLSCEASGFTFSHYGMHWVRQAPGKGLEWVAVIWYDGIMKNYIESVKGRFTISRDNSKNTLYLQMNRLRAEDTAVYYCARDGGFGELNYYGLDVWGQGTTVTVSSASTKGPSVFPLAPSSKSTSGGTAALGCLVKDYFPEPVTVSWNSGALTSGVHTFPAVLQSSGLYSLSSVVTVPSSSLGTQTYICNVNHKPSNTKVDKKVEPKSCDKTHTCPPCPAPELLGGPSVFLFPPKPKDTLMISRTPEVTCVVVDVSHEDPEVKFNWYVDGVEVHNAKTKPREEQYNSTYRVVSVLTVLHQDWLNGKEYKCKVSNKALPAPIEKTISKAKGQPREPQVYTLPPSREEMTKNQVSLTCLVKGFYPSDIAVEWESNGQPENNYKTTPPVLDSDGSFFLYSKLTVDKSRWQQGNVFSCSVMHEALHNHYTQKSLSLSPGK

SEQ ID NO: 262 - protein, 452 aa, Artificial sequence
  Heavy chain
QVQLVESGGGVVQPGTSLRLSCVASGFTFSNDGMHWVRQAPGMGLEWVAIMWFDGGSKYYADSVKGRFTISRDNSKNTLYLQMNNLRAEDTAVYYCARDHPHYLGSGSFDYWGQGTLVTVSSASTKGPSVFPLAPSSKSTSGGTAALGCLVKDYFPEPVTVSWNSGALTSGVHTFPAVLQSSGLYSLSSVVTVPSSSLGTQTYICNVNHKPSNTKVDKKVEPKSCDKTHTCPPCPAPELLGGPSVFLFPPKPKDTLMISRTPEVTCVVVDVSHEDPEVKFNWYVDGVEVHNAKTKPREEQYNSTYRVVSVLTVLHQDWLNGKEYKCKVSNKALPAPIEKTISKAKGQPREPQVYTLPPSREEMTKNQVSLTCLVKGFYPSDIAVEWESNGQPENNYKTTPPVLDSDGSFFLYSKLTVDKSRWQQGNVFSCSVMHEALHNHYTQKSLSLSPGK

SEQ ID NO: 263 - protein, 453 aa, Artificial sequence
  Heavy chain
QVQLVESGGDVVQPGRSLRLSCEASGFTFSHYGMHWVRQAPGKGLEWVAVVWYDGIKKYYVESVKGRFTISRDNSKNTLYLQMNRLRAEDTAVYYCARDGGFGELNYYGLDVWGQGTTVTVSSASTKGPSVFPLAPSSKSTSGGTAALGCLVKDYFPEPVTVSWNSGALTSGVHTFPAVLQSSGLYSLSSVVTVPSSSLGTQTYICNVNHKPSNTKVDKKVEPKSCDKTHTCPPCPAPELLGGPSVFLFPPKPKDTLMISRTPEVTCVVVDVSHEDPEVKFNWYVDGVEVHNAKTKPREEQYNSTYRVVSVLTVLHQDWLNGKEYKCKVSNKALPAPIEKTISKAKGQPREPQVYTLPPSREEMTKNQVSLTCLVKGFYPSDIAVEWESNGQPENNYKTTPPVLDSDGSFFLYSKLTVDKSRWQQGNVFSCSVMHEALHNHYTQKSLSLSPGK

SEQ ID NO: 264 - protein, 449 aa, Artificial sequence
  Heavy chain
QVQLQQSGPGLVKPSQTLSLTCAISGDSVSSTSAVWNWIRQSPSRGLEWLGRTCYRSKWYNDYAVSVKSRITITPDTSKNQFSLRLNPVTPEDTAVYYCARGDFRFDSWGQGTLVTVSSASTKGPSVFPLAPSSKSTSGGTAALGCLVKDYFPEPVTVSWNSGALTSGVHTFPAVLQSSGLYSLSSVVTVPSSSLGTQTYICNVNHKPSNTKVDKKVEPKSCDKTHTCPPCPAPELLGGPSVFLFPPKPKDTLMISRTPEVTCVVVDVSHEDPEVKFNWYVDGVEVHNAKTKPREEQYNSTYRVVSVLTVLHQDWLNGKEYKCKVSNKALPAPIEKTISKAKGQPREPQVYTLPPSREEMTKNQVSLTCLVKGFYPSDIAVEWESNGQPENNYKTTPPVLDSDGSFFLYSKLTVDKSRWQQGNVFSCSVMHEALHNHYTQKSLSLSPGK

SEQ ID NO: 265 - protein, 453 aa, Artificial sequence
  Heavy chain
QVQLVESGGGVVQPGRSLRLSCEASGFTFSHYGMHWVRQAPGKGLEWVAVIWYDGIKTYYVESVKGRFTISRDNSKNTLNLQMNRLRAEDTAVYYCARDGGFGESNYYGLDVWGQGTTVTVSSASTKGPSVFPLAPSSKSTSGGTAALGCLVKDYFPEPVTVSWNSGALTSGVHTFPAVLQSSGLYSLSSVVTVPSSSLGTQTYICNVNHKPSNTKVDKKVEPKSCDKTHTCPPCPAPELLGGPSVFLFPPKPKDTLMISRTPEVTCVVVDVSHEDPEVKFNWYVDGVEVHNAKTKPREEQYNSTYRVVSVLTVLHQDWLNGKEYKCKVSNKALPAPIEKTISKAKGQPREPQVYTLPPSREEMTKNQVSLTCLVKGFYPSDIAVEWESNGQPENNYKTTPPVLDSDGSFFLYSKLTVDKSRWQQGNVFSCSVMHEALHNHYTQKSLSLSPGK

SEQ ID NO: 266 - protein, 448 aa, Artificial sequence
  Heavy chain
QVQLQESGPGLVKPSETLSLTCAVSGYSISSGYFWAWIRQPPGKGLEWIGSIYHSGRTHYNPSLKSRVIISLDTSKNQFSLKLRSVTAADSAVYYCAREGYASGSYYWGQGTLVTVSSASTKGPSVFPLAPSSKSTSGGTAALGCLVKDYFPEPVTVSWNSGALTSGVHTFPAVLQSSGLYSLSSVVTVPSSSLGTQTYICNVNHKPSNTKVDKKVEPKSCDKTHTCPPCPAPELLGGPSVFLFPPKPKDTLMISRTPEVTCVVVDVSHEDPEVKFNWYVDGVEVHNAKTKPREEQYNSTYRVVSVLTVLHQDWLNGKEYKCKVSNKALPAPIEKTISKAKGQPREPQVYTLPPSREEMTKNQVSLTCLVKGFYPSDIAVEWESNGQPENNYKTTPPVLDSDGSFFLYSKLTVDKSRWQQGNVFSCSVMHEALHNHYTQKSLSLSPGK

SEQ ID NO: 267 - protein, 451 aa, Artificial sequence
  Heavy chain
QVQLVESGGGVVQPGRSLRLSCATSGFIFSSYGMHWVRQAPGKGLDWVAVIWYDGSNKYYADSVKGRFTISRDNSKNTLYLQMNSLRVEDTAVYYCARETSSWYVGYLQHWGQGTLVTVSSASTKGPSVFPLAPSSKSTSGGTAALGCLVKDYFPEPVTVSWNSGALTSGVHTFPAVLQSSGLYSLSSVVTVPSSSLGTQTYICNVNHKPSNTKVDKKVEPKSCDKTHTCPPCPAPELLGGPSVFLFPPKPKDTLMISRTPEVTCVVVDVSHEDPEVKFNWYVDGVEVHNAKTKPREEQYNSTYRVVSVLTVLHQDWLNGKEYKCKVSNKALPAPIEKTISKAKGQPREPQVYTLPPSREEMTKNQVSLTCLVKGFYPSDIAVEWESNGQPENNYKTTPPVLDSDGSFFLYSKLTVDKSRWQQGNVFSCSVMHEALHNHYTQKSLSLSPGK

SEQ ID NO: 268 - protein, 448 aa, Artificial sequence
  Heavy chain
QVQLQESGPGLVKPSETLSLTCAVSGYSINSGYFWAWIRQPPGMGLEWIGSIYHSGRTHYNPSLKSRVIISLDTSKNQFSLKLRSVTAADSAVYYCAREGYASGSYYWGQGTLVTVSSASTKGPSVFPLAPSSKSTSGGTAALGCLVKDYFPEPVTVSWNSGALTSGVHTFPAVLQSSGLYSLSSVVTVPSSSLGTQTYICNVNHKPSNTKVDKKVEPKSCDKTHTCPPCPAPELLGGPSVFLFPPKPKDTLMISRTPEVTCVVVDVSHEDPEVKFNWYVDGVEVHNAKTKPREEQYNSTYRVVSVLTVLHQDWLNGKEYKCKVSNKALPAPIEKTISKAKGQPREPQVYTLPPSREEMTKNQVSLTCLVKGFYPSDIAVEWESNGQPENNYKTTPPVLDSDGSFFLYSKLTVDKSRWQQGNVFSCSVMHEALHNHYTQKSLSLSPGK

SEQ ID NO: 269 - protein, 453 aa, Artificial sequence
  Heavy chain
QVQLVESGGGVVQPGRSLRLSCAASGFTFSHYGMHWVRQAPGKGLEWVAVIWYDGIKKNYVESVKGRFTISRDNSKNTLNLQMNRLRAEDTAVYYCARDGGFGESNYYGLDVWGQGTTVTVSSASTKGPSVFPLAPSSKSTSGGTAALGCLVKDYFPEPVTVSWNSGALTSGVHTFPAVLQSSGLYSLSSVVTVPSSSLGTQTYICNVNHKPSNTKVDKKVEPKSCDKTHTCPPCPAPELLGGPSVFLFPPKPKDTLMISRTPEVTCVVVDVSHEDPEVKFNWYVDGVEVHNAKTKPREEQYNSTYRVVSVLTVLHQDWLNGKEYKCKVSNKALPAPIEKTISKAKGQPREPQVYTLPPSREEMTKNQVSLTCLVKGFYPSDIAVEWESNGQPENNYKTTPPVLDSDGSFFLYSKLTVDKSRWQQGNVFSCSVMHEALHNHYTQKSLSLSPGK

SEQ ID NO: 270 - protein, 213 aa, Artificial sequence
  Light chain
EIVLTQSPATLSLSPGERATLSCRASQSVGSYLAWYQQKPGQAPSLLIYDASNRATGIPARFSGSGSGTDFTLTISSLEPEDFAVYYCQQRTNWYTFGQGTKLEIKRTVAAPSVFIFPPSDEQLKSGTASVVCLLNNFYPREAKVQWKVDNALQSGNSQESVTEQDSKDSTYSLSSTLTLSKADYEKHKVYACEVTHQGLSSPVTKSFNRGEC

SEQ ID NO: 271 - protein, 215 aa, Artificial sequence
  Light chain
DIQMTQSPSTLSASVGDRVTITCRASQSIGNWLAWYQQKPGKAPKLLIYKASSLESGVPSRFSGSGSGTEFTLTISSLQPDDFATYYCQQYDSYSPITFGQGTRLEIKRTVAAPSVFIFPPSDEQLKSGTASVVCLLNNFYPREAKVQWKVDNALQSGNSQESVTEQDSKDSTYSLSSTLTLSKADYEKHKVYACEVTHQGLSSPVTKSFNRGEC

SEQ ID NO: 272 - protein, 214 aa, Artificial sequence
  Light chain
DIQMTQSPSSLSASLGDRVTITCRATQGISNYLAWYQQKPGKVPNLLIYAASTLQSGVPSRFSGSGSGTDLTLTISSLQPEDVATYYCQKCNSAPRTFGQGTKVEIKRTVAAPSVFIFPPSDEQLKSGTASVVCLLNNFYPREAKVQWKVDNALQSGNSQESVTEQDSKDSTYSLSSTLTLSKADYEKHKVYACEVTHQGLSSPVTKSFNRGEC

SEQ ID NO: 273 - protein, 215 aa, Artificial sequence
  Light chain
DIQMTQSPSSLSASVGERVTITCRASQNINSYLSWYQQKPGKAPKLLIYAASSLQNGVPSRFSGSGSGTDFTLTISSLQPEDFATYYCQQSFSTPPITFGQGTRLEIKRTVAAPSVFIFPPSDEQLKSGTASVVCLLNNFYPREAKVQWKVDNALQSGNSQESVTEQDSKDSTYSLSSTLTLSKADYEKHKVYACEVTHQGLSSPVTKSFNRGEC

SEQ ID NO: 274 - protein, 215 aa, Artificial sequence
  Light chain
DIQMTQSPSSLSASVGDRVTITCRASQNINSYLHWYQQKPGKAPKLLIYAASSLQSGVPSRFSGSGSGTDFTLTISSLQPEDFAIYYCQQSYSIPPITFGQGTRLEIKRTVAAPSVFIFPPSDEQLKSGTASVVCLLNNFYPREAKVQWKVDNALQSGNSQESVTEQDSKDSTYSLSSTLTLSKADYEKHKVYACEVTHQGLSSPVTKSFNRGEC

SEQ ID NO: 275 - protein, 214 aa, Artificial sequence
  Light chain
DIQMTQSPSSLSASVGDRVTITCRASQGISHFLAWYQQKPGKVPKLLIYAASTLQSGVPSRFSGSGSGTDFTLTISSLQPEDVATYYCQKFNSAPLTFGGGTKVEIKRTVAAPSVFIFPPSDEQLKSGTASVVCLLNNFYPREAKVQWKVDNALQSGNSQESVTEQDSKDSTYSLSSTLTLSKADYEKHKVYACEVTHQGLSSPVTKSFNRGEC

SEQ ID NO: 276 - protein, 214 aa, Artificial sequence
  Light chain
DIQMTQSPSTLSASVGDRVTITCRASQSISNWLAWYQQKPGKAPKVLIYKASSLESGVPSRFSGSGSGTEFTLTINSLQPDDFATYYCQQYDSYSITFGQGTRLEIKRTVAAPSVFIFPPSDEQLKSGTASVVCLLNNFYPREAKVQWKVDNALQSGNSQESVTEQDSKDSTYSLSSTLTLSKADYEKHKVYACEVTHQGLSSPVTKSFNRGEC

SEQ ID NO: 277 - protein, 215 aa, Artificial sequence
  Light chain
QVVMTQSPATLSVSPGERATLSCRASQSVSSKLAWYQQKPGQAPRLIIYGASTRATGIPARFSGSGSGTEFTLTISSLQSEDFAVYYCQQYDNWPPITFGQGTRLEIKRTVAAPSVFIFPPSDEQLKSGTASVVCLLNNFYPREAKVQWKVDNALQSGNSQESVTEQDSKDSTYSLSSTLTLSKADYEKHKVYACEVTHQGLSSPVTKSFNRGEC

SEQ ID NO: 278 - protein, 215 aa, Artificial sequence
  Light chain
DIQMTQSPSTLSASVGDRVTITCRASQSIGHWLAWYQQKPGKAPKLLIYKASSLESGVPSRFRGSGSGTEFTLTISSLQPDDFATYYCQQYSSYSPITFGQGSRLEIKRTVAAPSVFIFPPSDEQLKSGTASVVCLLNNFYPREAKVQWKVDNALQSGNSQESVTEQDSKDSTYSLSSTLTLSKADYEKHKVYACEVTHQGLSSPVTKSFNRGEC

SEQ ID NO: 279 - protein, 215 aa, Artificial sequence
  Light chain
EIVMTQSPATLSVSPGERATLSCRASQSVSSNLAWYQQKPGQAPRLLIYGASTRATGIPARFSGSGSGTEFTLTISSLQSEDFAVYYCQQYNNWPPITFGQGTRLEIKRTVAAPSVFIFPPSDEQLKSGTASVVCLLNNFYPREAKVQWKVDNALQSGNSQESVTEQDSKDSTYSLSSTLTLSKADYEKHKVYACEVTHQGLSSPVTKSFNRGEC

SEQ ID NO: 280 - protein, 215 aa, Artificial sequence
  Light chain
DIQMTQSPSSLSASVGDRVTITCRASQSINSYLHWYQQKPGKAPKLLIYAASSLQSGVPSRFSGSGSGTDFTLTISSLQPEDFATYYCQQSYSTPPITFGQGTRLEIKRTVAAPSVFIFPPSDEQLKSGTASVVCLLNNFYPREAKVQWKVDNALQSGNSQESVTEQDSKDSTYSLSSTLTLSKADYEKHKVYACEVTHQGLSSPVTKSFNRGEC

SEQ ID NO: 281 - protein, 214 aa, Artificial sequence
  Light chain
DIQLTQSPSFLSASVGDRVTITCRASQGINSYLGWYQRKPGKAPKLLIYIASTLQSGVPSRFSGSGSGTEFTLTISSLQPEDFATYYCQQLNSYPYTFGQGTKLEIKRTVAAPSVFIFPPSDEQLKSGTASVVCLLNNFYPREAKVQWKVDNALQSGNSQESVTEQDSKDSTYSLSSTLTLSKADYEKHKVYACEVTHQGLSSPVTKSFNRGEC

SEQ ID NO: 282 - protein, 214 aa, Artificial sequence
  Light chain
DIQLTQSPSFLSASVGDRVTITCRASQGISSYLGWYQQKPGKAPKLLIYVASTLQSGVPSRFSGSGSGTEFTLTISSLQPEDFATYYCQQLNSYPYTFGQGTKLEIKRTVAAPSVFIFPPSDEQLKSGTASVVCLLNNFYPREAKVQWKVDNALQSGNSQESVTEQDSKDSTYSLSSTLTLSKADYEKHKVYACEVTHQGLSSPVTKSFNRGEC

SEQ ID NO: 283 - protein, 215 aa, Artificial sequence
  Light chain
EIVLTQFPGTLSLSPGERATLSCRSSQSVSSSYLAWYQQKPGQAPRLLISGASSRATGIPDRFSGSGSGTDFTLTISRLEPEDFAVYYCQQYGSSPRTFGQGTKVEIKRTVAAPSVFIFPPSDEQLKSGTASVVCLLNNFYPREAKVQWKVDNALQSGNSQESVTEQDSKDSTYSLSSTLTLSKADYEKHKVYACEVTHQGLSSPVTKSFNRGEC

SEQ ID NO: 284 - protein, 214 aa, Artificial sequence
  Light chain
DIQLTQSPSFLSASVGDRVTITCRASQGISSYLGWYQQKPGKAPKLLIYIASTLQSGVPSRFSGSGSGTEFTLTISSLQPEDFATYYCQQLNSYPYTFGQGTKLEIKRTVAAPSVFIFPPSDEQLKSGTASVVCLLNNFYPREAKVQWKVDNALQSGNSQESVTEQDSKDSTYSLSSTLTLSKADYEKHKVYACEVTHQGLSSPVTKSFNRGEC

SEQ ID NO: 285 - protein, 214 aa, Artificial sequence
  Light chain
EIVLTQSPATLSLSPGERATLSCRASQSVSSYLAWYQQKPGQAPRLLIYDASNRATGIPARFSGSGSGTDFTLTISSLQAEDVAVYYCQQYYSTPYTFGQGTKLEIKRTVAAPSVFIFPPSDEQLKSGTASVVCLLNNFYPREAKVQWKVDNALQSGNSQESVTEQDSKDSTYSLSSTLTLSKADYEKHKVYACEVTHQGLSSPVTKSFNRGEC

SEQ ID NO: 286 - protein, 214 aa, Artificial sequence
  Light chain
DIQLTQSPSFLSASVGDRVTITCRASQGISSYLAWYQQKPGKAPKLLIYAASTLQSGVPSRFSGSGSGTEFTLTISSLQPEDFATYYCQQVKIYPLTFGGGTKVEIKRTVAAPSVFIFPPSDEQLKSGTASVVCLLNNFYPREAKVQWKVDNALQSGNSQESVTEQDSKDSTYSLSSTLTLSKADYEKHKVYACEVTHQGLSSPVTKSFNRGEC

SEQ ID NO: 287 - protein, 214 aa, Artificial sequence
  Light chain
EIVMTQSPATLSVSPGERATLSCRSSQSVNNYLAWFQQKPGQAPRLLIYDSSTRATGIPARFSGSGSGTEFTLTISSLQSEDFAFYFCQQYENWPLTFGGGTKVEIKRTVAAPSVFIFPPSDEQLKSGTASVVCLLNNFYPREAKVQWKVDNALQSGNSQESVTEQDSKDSTYSLSSTLTLSKADYEKHKVYACEVTHQGLSSPVTKSFNRGEC

SEQ ID NO: 288 - protein, 214 aa, Artificial sequence
  Light chain
EIVMTQSPATLSVSPGERVSLSCRASQSVNGNVAWYQQKPGQAPRLLIYAASTRATGIPARFSGSGSGTESTLTISSLQSEDCAVYYCQQYNNWPSTFGPGTKLEVTRTVAAPSVFIFPPSDEQLKSGTASVVCLLNNFYPREAKVQWKVDNALQSGNSQESVTEQDSKDSTYSLSSTLTLSKADYEKHKVYACEVTHQGLSSPVTKSFNRGEC

SEQ ID NO: 289 - protein, 214 aa, Artificial sequence
  Light chain
EIVMTQSPATLSVSPGERATLSCRSSQSVNSYLAWFQQKPGQAPRLLIYDSSTRATGIPARFSGSGSGTEFTLTISSLQSEDFAFYFCQQYENWPLTFGGGTKVEIKRTVAAPSVFIFPPSDEQLKSGTASVVCLLNNFYPREAKVQWKVDNALQSGNSQESVTEQDSKDSTYSLSSTLTLSKADYEKHKVYACEVTHQGLSSPVTKSFNRGEC

SEQ ID NO: 290 - protein, 451 aa, Artificial sequence
  Heavy chain
QVQLQQSGSELKKPGASVKVSCKASGYTFTNYGMNWVKQAPGQGLKWMGWINTYTGEPTYTDDFKGRFAFSLDTSVSTAYLQISSLKADDTAVYFCARGGFGSSYWYFDVWGQGSLVTVSSASTKGPSVFPLAPSSKSTSGGTAALGCLVKDYFPEPVTVSWNSGALTSGVHTFPAVLQSSGLYSLSSVVTVPSSSLGTQTYICNVNHKPSNTKVDKRVEPKSCDKTHTCPPCPAPELLGGPSVFLFPPKPKDTLMISRTPEVTCVVVDVSHEDPEVKFNWYVDGVEVHNAKTKPREEQYNSTYRVVSVLTVLHQDWLNGKEYKCKVSNKALPAPIEKTISKAKGQPREPQVYTLPPSREEMTKNQVSLTCLVKGFYPSDIAVEWESNGQPENNYKTTPPVLDSDGSFFLYSKLTVDKSRWQQGNVFSCSVMHEALHNHYTQKSLSLSPGK

SEQ ID NO: 291 - protein, 214 aa, Artificial sequence
  Light chain
DIQLTQSPSSLSASVGDRVSITCKASQDVSIAVAWYQQKPGKAPKLLIYSASYRYTGVPDRFSGSGSGTDFTLTISSLQPEDFAVYYCQQHYITPLTFGAGTKVEIKRTVAAPSVFIFPPSDEQLKSGTASVVCLLNNFYPREAKVQWKVDNALQSGNSQESVTEQDSKDSTYSLSSTLTLSKADYEKHKVYACEVTHQGLSSPVTKSFNRGEC

SEQ ID NO: 292 - protein, 330 aa, Artificial sequence
  Heavy chain constant region
ASTKGPSVFPLAPSSKSTSGGTAALGCLVKDYFPEPVTVSWNSGALTSGVHTFPAVLQSSGLYSLSSVVTVPSSSLGTQTYICNVNHKPSNTKVDKKVEPKSCDKTHTCPPCPAPELLGGPSVFLFPPKPKDTLMISRTPEVTCVVVDVSHEDPEVKFNWYVDGVEVHNAKTKPREEQYNSTYRVVSVLTVLHQDWLNGKEYKCKVSNKALPAPIEKTISKAKGQPREPQVYTLPPSREEMTKNQVSLTCLVKGFYPSDIAVEWESNGQPENNYKTTPPVLDSDGSFFLYSKLTVDKSRWQQGNVFSCSVMHEALHNHYTQKSLSLSPGK

SEQ ID NO: 293 - protein, 107 aa, Artificial sequence [sequence omitted]